European Patent Application EP 4 748 937 A1, published May 27, 2026. Title: 외래 리보스 포스페이트 디포스포키나제가 도입된 미생물 및 이를 이용한 L-트립토판 생산 방법. Applicant: 씨제이제일제당 주식회사. The sequence listing filed with the application follows.

SEQUENCE LISTING (27 sequences)

SEQ ID NO: 1 - protein, 317 aa, Bacillus subtilis
MSNQYGDKNLKIFSLNSNPELAKEIADIVGVQLGKCSVTRFSDGEVQINIEESIRGCDCYIIQSTSDPVNEHIMELLIMVDALKRASAKTINIVIPYYGYARQDRKARSREPITAKLFANLLETAGATRVIALDLHAPQIQGFFDIPIDHLMGVPILGEYFEGKNLEDIVIVSPDHGGVTRARKLADRLKAPIAIIDKRRPRPNVAEVMNIVGNIEGKTAILIDDIIDTAGTITLAANALVENGAKEVYACCTHPVLSGPAVERINNSTIKELVVTNSIKLPEEKKIERFKQLSVGPLLAEAIIRVHEQQSVSYLFS

SEQ ID NO: 2 - DNA, 954 bp, Bacillus subtilis
  source 1..954: mol_type = genomic DNA
atgtctaatcaatacggagataagaatttaaagattttttctttgaattcgaatccagagcttgcaaaagaaatcgcagatatagttggagttcaattagggaaatgttctgtcacaagatttagtgacggggaagtccaaattaatatcgaagaaagtattcgcggatgtgattgttacatcatccagtctacaagtgaccccgttaacgagcatattatggaactgctgattatggtagatgcgttaaaacgcgcttctgcaaaaacgattaacattgttattccttattacggttatgcgcgtcaagacagaaaagcaagatcccgtgagccaatcacagctaaacttttcgctaacctgcttgaaacagccggtgcgactcgtgtgattgcacttgacctgcatgcgccgcaaattcaaggattctttgatataccgattgaccacttaatgggtgttccgattttaggagaatattttgaaggcaaaaatcttgaagatatcgtcattgtttcaccagaccatggcggtgtgacacgtgcccgcaaactggctgaccgactaaaagcgccaattgcgattatcgataaacgccgtccgcgtccaaacgtggcggaagtcatgaatattgtaggtaacatcgaagggaagactgctatcctcatcgatgacattattgatactgcaggtacgattacacttgctgctaatgcgctcgttgaaaacggagcgaaagaagtatatgcatgctgtacacaccctgtactatcaggccctgcggttgaacggattaataattcaacaattaaagagcttgttgtgacaaacagcatcaagcttcctgaagaaaagaaaattgaacgctttaagcagctttcagtcggaccgcttctggccgaagcgattattcgcgttcatgagcagcaatcagtcagctatctgttcagctaa

SEQ ID NO: 3 - protein, 326 aa, Mycobacterium smegmatis
MATDWTDNRKNLMLFAGRAHPELADQVAKELDVAVTAQTARDFANGEIFVRFDESVRGCDAFVLQSHPAPLNQWLMEQLIMIDALKRGSAKRITAILPFYPYARQDKKHRGREPISARLVADLLKTAGADRIVSVDLHTDQIQGFFDGPVDHMRAQKLLTGYIGEHYADEDMVVVSPDSGRVRVAEKWADSLGGVPLAFIHKTRDPLVPNQVKSNRVVGDVKGKTCILTDDMIDTGGTIAGAVNLLREDGAKDVIIAATHGVLSDPAPQRLAECGAREVIVTNTLPITEDKRFPQLTVLSIAPLLANTIRAVFENGSVTGLFDGSA

SEQ ID NO: 4 - DNA, 981 bp, Mycobacterium smegmatis
  source 1..981: mol_type = genomic DNA
gtggccacggactggaccgacaatcgcaaaaacttgatgctgttcgcgggtcgcgcgcaccccgagctggctgaccaagttgccaaagaactcgacgtggccgtcaccgcgcaaacggcacgggatttcgccaacggtgagatcttcgtccgcttcgacgaatccgtccgtggctgtgacgcattcgtgctgcagagccatccggcgccgctgaaccagtggctcatggaacagctgatcatgatcgacgcgctcaagcgtggcagcgccaagcgcatcaccgcgatcctgccgttctatccctacgcccggcaggacaagaagcaccgcggccgcgaacccatctcggcacgcctcgtcgcggacctgctcaagaccgcgggcgccgaccgcatcgtgtcggtcgacctgcacaccgaccagatccagggcttcttcgacggcccggtggaccacatgcgcgcgcagaagctgctcaccggctacatcggcgagcactacgccgacgaggacatggtggtggtgtcccccgattcgggccgcgtgcgtgtcgccgagaagtgggccgactcgctgggcggtgttccgctggccttcatccacaagacgcgtgacccgctggtccccaaccaggtcaagtcgaaccgcgtcgtgggtgacgtcaagggcaagacctgcatcctcaccgacgacatgatcgacacgggcggcacgatcgccggcgcggtcaacctgctgcgtgaggacggcgccaaggacgtcatcatcgccgcgacgcacggcgtgctgtcggatcccgccccgcagcggctcgccgagtgcggcgcacgcgaggtgatcgtcaccaacacgctgcccatcaccgaggacaagcgcttcccgcagctcacggtgctctccatcgcaccgcttctggccaacaccatccgggccgtgttcgagaacggttcggtgacaggactgttcgacgggtctgcataa

SEQ ID NO: 5 - protein, 315 aa, Escherichia coli
MPDMKLFAGNATPELAQRIANRLYTSLGDAAVGRFSDGEVSVQINENVRGGDIFIIQSTCAPTNDNLMELVVMVDALRRASAGRITAVIPYFGYARQDRRVRSARVPITAKVVADFLSSVGVDRVLTVDLHAEQIQGFFDVPVDNVFGSPILLEDMLQLNLDNPIVVSPDIGGVVRARAIAKLLNDTDMAIIDKRRPRANVSQVMHIIGDVAGRDCVLVDDMIDTGGTLCKAAEALKERGAKRVFAYATHPIFSGNAANNLRNSVIDEVVVCDTIPLSDEIKSLPNVRTLTLSGMLAEAIRRISNEESISAMFEH

SEQ ID NO: 6 - DNA, 948 bp, Escherichia coli
  source 1..948: mol_type = genomic DNA
atgcctgatatgaagctttttgctggtaacgccaccccggaactagcacaacgtattgccaaccgcctgtacacttcactcggcgacgccgctgtaggtcgctttagcgatggcgaagtcagcgtacaaattaatgaaaatgtacgcggtggtgatattttcatcatccagtccacttgtgcccctactaacgacaacctgatggaattagtcgttatggttgatgccctgcgtcgtgcttccgcaggtcgtatcaccgctgttatcccctactttggctatgcgcgccaggaccgtcgcgtccgttccgctcgtgtaccaatcactgcgaaagtggttgcagacttcctctccagcgtcggtgttgaccgtgtgctgacagtggatctgcacgctgaacagattcagggtttcttcgacgttccggttgataacgtatttggtagcccgatcctgctggaagacatgctgcagctgaatctggataacccaattgtggtttctccggacatcggcggcgttgtgcgtgcccgcgctatcgctaagctgctgaacgataccgatatggcaatcatcgacaaacgtcgtccgcgtgcgaacgtttcacaggtgatgcatatcatcggtgacgttgcaggtcgtgactgcgtactggtcgatgatatgatcgacactggcggtacgctgtgtaaagctgctgaagctctgaaagaacgtggtgctaaacgtgtatttgcgtacgcgactcacccgatcttctctggcaacgcggcgaacaacctgcgtaactctgtaattgatgaagtcgttgtctgcgataccattccgctgagcgatgaaatcaaatcactgccgaacgtgcgtactctgaccctgtcaggtatgctggccgaagcgattcgtcgtatcagcaacgaagaatcgatctctgccatgttcgaacactaa

SEQ ID NO: 7 - protein, 325 aa, Corynebacterium glutamicum
MTAHWKQNQKNLMLFSGRAHPELAEAVAKELDVNVTPMTARDFANGEIYVRFEESVRGSDCFVLQSHTQPLNKWLMEQLLMIDALKRGSAKRITAILPFYPYARQDKKHRGREPISARLIADLMLTAGADRIVSVDLHTDQIQGFFDGPVDHMHAMPILTDHIKENYNLDNICVVSPDAGRVKVAEKWANTLGDAPMAFVHKTRSTEVANQVVANRVVGDVDGKDCVLLDDMIDTGGTIAGAVGVLKKAGAKSVVIACTHGVFSDPARERLSACGAEEVITTDTLPQSTEGWSNLTVLSIAPLLARTINEIFENGSVTTLFEGEA

SEQ ID NO: 8 - DNA, 978 bp, Corynebacterium glutamicum
  source 1..978: mol_type = genomic DNA
atgactgctcactggaaacaaaaccaaaagaacctcatgctgttttcgggtcgtgcgcacccagaactggcagaagctgtagctaaagagctcgacgtcaacgtcaccccaatgacggcacgcgatttcgccaacggtgagatctacgtccgcttcgaggaatcagttcgtggctccgactgcttcgtcctgcagtcccacacccagcctctcaacaagtggctcatggaacagctgctgatgatcgacgctttgaagcgtggttccgcaaagcgcatcaccgcgatcctgccgttctacccttacgcccgccaggacaagaagcaccgcggccgcgagccaatttctgctcgcctcatcgccgacctcatgctcaccgctggcgcggaccgtatcgtgtccgtggacttgcacaccgatcagatccagggcttcttcgacggcccagtcgatcacatgcacgccatgccgatcctcaccgatcacatcaaggaaaactacaacctggacaacatctgcgtggtctcccctgacgcaggtcgcgtgaaggttgcagagaagtgggctaacaccttgggcgatgccccaatggcgttcgtgcacaagacccgctccaccgaggtagcaaaccaggttgtcgccaaccgcgtcgtcggtgacgtcgacggcaaggactgcgtgcttctcgacgacatgatcgacactggcggcaccatcgccggcgctgtgggcgtcctgaagaaggctggcgcaaagtcagtcgtcatcgcctgcacccacggtgtgttctctgacccagcccgcgagcgcctgtctgcatgcggtgctgaagaagtcatcaccaccgacaccctgccacagtccaccgagggctggagcaacctgaccgttttgtcgatcgcaccgctgctggctcgcaccatcaacgagatcttcgaaaacggctccgtcaccaccctcttcgagggcgaggcctaa

SEQ ID NO: 9 - DNA, 38 bp, synthetic construct
  source 1..38: mol_type = other DNA
aacgacggccagtgaattctcgttggccattacctcat

SEQ ID NO: 10 - DNA, 45 bp, synthetic construct
  source 1..45: mol_type = other DNA
ctgtttagtactaaaccggaagggccttatctgccacacccacaa

SEQ ID NO: 11 - DNA, 45 bp, synthetic construct
  source 1..45: mol_type = other DNA
cggtttagtactaaacaggaagagcctaaaaacggaagagccact

SEQ ID NO: 12 - DNA, 39 bp, synthetic construct
  source 1..39: mol_type = other DNA
ttgcatgcctgcaggtcgacggaagactatccaaggtgg

SEQ ID NO: 13 - DNA, 40 bp, synthetic construct
  source 1..40: mol_type = other DNA
taaggcccttccggtttagtagaaacatcccagcgctact

SEQ ID NO: 14 - DNA, 40 bp, synthetic construct
  source 1..40: mol_type = other DNA
tctccgtattgattagacatgagtgtttcctttcgttggg

SEQ ID NO: 15 - DNA, 40 bp, synthetic construct
  source 1..40: mol_type = other DNA
cccaacgaaaggaaacactcatgtctaatcaatacggaga

SEQ ID NO: 16 - DNA, 40 bp, synthetic construct
  source 1..40: mol_type = other DNA
ttaggctcttcctgtttagtttagctgaacagatagctga

SEQ ID NO: 17 - DNA, 18 bp, synthetic construct
  source 1..18: mol_type = other DNA
gttcggcttggattatgg

SEQ ID NO: 18 - DNA, 18 bp, synthetic construct
  source 1..18: mol_type = other DNA
catcaacaacagccttca

SEQ ID NO: 19 - DNA, 40 bp, synthetic construct
  source 1..40: mol_type = other DNA
tcggtccagtccgtggccacgagtgtttcctttcgttggg

SEQ ID NO: 20 - DNA, 40 bp, synthetic construct
  source 1..40: mol_type = other DNA
cccaacgaaaggaaacactcgtggccacggactggaccga

SEQ ID NO: 21 - DNA, 40 bp, synthetic construct
  source 1..40: mol_type = other DNA
ttaggctcttcctgtttagtttatgcagacccgtcgaaca

SEQ ID NO: 22 - DNA, 40 bp, synthetic construct
  source 1..40: mol_type = other DNA
aaaagcttcatatcaggcatgagtgtttcctttcgttggg

SEQ ID NO: 23 - DNA, 40 bp, synthetic construct
  source 1..40: mol_type = other DNA
cccaacgaaaggaaacactcatgcctgatatgaagctttt

SEQ ID NO: 24 - DNA, 40 bp, synthetic construct
  source 1..40: mol_type = other DNA
ttaggctcttcctgtttagtttagtgttcgaacatggcag

SEQ ID NO: 25 - DNA, 40 bp, synthetic construct
  source 1..40: mol_type = other DNA
tgtttccagtgagcagtcatgagtgtttcctttcgttggg

SEQ ID NO: 26 - DNA, 40 bp, synthetic construct
  source 1..40: mol_type = other DNA
cccaacgaaaggaaacactcatgactgctcactggaaaca

SEQ ID NO: 27 - DNA, 40 bp, synthetic construct
  source 1..40: mol_type = other DNA
ttaggctcttcctgtttagtttaggcctcgccctcgaaga